European Patent Specification EP 3 457 139 B1, published August 5, 2026. Title: ANTIBODY-LIKE PEPTIDES FOR QUANTIFYING THERAPEUTIC ANTIBODIES. Applicant: PROMISE ADVANCED PROTEOMICS. The sequence listing filed with the application follows.

SEQUENCE LISTING (119 sequences)

SEQ ID NO: 1 - protein, 218 aa, Artificial Sequence
  >SEQID1
EVQLVESGGGLVQPGGSLRLSCAASGFNIKDTYIHWVRQAPGKGLEWLGVIWSGGNTDYNTPFTSRLSINKDNSKSTAYLQMNSLRAEDTAVYYCSRWGGDGFYAMDYWGQGTLVTVSSASTKGPSVFPLAPSSKSTSGGTAALGCLVKDYFPEPVTVSWNSGALTSGVHTFPAVLQSSGLYSLSSVVTVPSSSLGTQTYICNVNHKPSNTKVDKKVE

SEQ ID NO: 2 - protein, 219 aa, Artificial Sequence
  >SEQID2
EVQLVESGGGLVQPGGSLRLSCAASGFNIKDTYIHWVRQAPGKGLEWVGWINTYTGEPTYAADFKRRFTFSLDTSKSTAYLQMNSLRAEDTAVYYCSRWGGDGFYAMDYWGQGTLVTVSSASTKGPSVFPLAPSSKSTSGGTAALGCLVKDYFPEPVTVSWNSGALTSGVHTFPAVLQSSGLYSLSSVVTVPSSSLGTQTYICNVNHKPSNTKVDKKVE

SEQ ID NO: 3 - protein, 238 aa, Artificial Sequence
  >SEQID3
KVDKKVEPKSCDKTHTCPPCPAPELLGGPSVFLFPPKPKDTLMISRTPEVTCVVVDVSHEDPEVKFNWYVDGVEVHNAKTKPREEQYNSTYRVVSVLTVLHQDWLNGKEYKCKVSNKALPAPIEKTISKAKGQPREPQVYTLPPCREEMTKNQVSLWCLVKGFYPSDIAVEWESNGQPENNYKTTPPVLDSDGSFFLYSKLTVDKSRWQQGNVFSCSVMHEALHNHYTQKSLSLSPGK

SEQ ID NO: 4 - protein, 238 aa, Artificial Sequence
  >SEQID4
KVDKKVEPKSCDKTHTCPPCPAPELLGGPSVFLFPPKPKDTLMISRTPEVTCVVVDVSHEDPEVKFNWYVDGVEVHNAKTKPREEQYNSTYRVVSVLTVLHQDWLNGKEYKCKVSNKALPAPIEKTISKAKGQPREPQVCTLPPSREEMTKNQVSLSCAVKGFYPSDIAVEWESNGQPENNYKTTPPVLDSDGSFFLVSKLTVDKSRWQQGNVFSCSVMHEALHNHYTQKSLSLSPGK

SEQ ID NO: 5 - protein, 214 aa, Artificial Sequence
  >SEQID5
DIQMTQSPSSLSASVGDRVTITCRASQDVNTAVAWYQQKPGKAPKLLIYSASFLYSGVPSRFSGSRSGTDFTLTISSLQPEDFATYYCQQHYTTPPTFGQGTKVEIKRTVAAPSVFIFPPSDEQLKSGTASVVCLLNNFYPREAKVQWKVDNALQSGNSQESVTEQDSKDSTYSLSSTLTLSKADYEKHKVYACEVTHQGLSSPVTKSFNRGEC

SEQ ID NO: 6 - protein, 449 aa, Artificial Sequence
  >SEQID6
EVQLVESGGGLVQPGGSLRLSCAASGFNIKDTYIHWVRQAPGKGLEWLGVIWSGGNTDYNTPFTSRLSINKDNSKSTAYLQMNSLRAEDTAVYYCSRWGGDGFYAMDYWGQGTLVTVSSASTKGPSVFPLAPSSKSTSGGTAALGCLVKDYFPEPVTVSWNSGALTSGVHTFPAVLQSSGLYSLSSVVTVPSSSLGTQTYICNVNHKPSNTKVDKKVEPKSCDKTHTCPPCPAPELLGGPSVFLFPPKPKDTLMISRTPEVTCVVVDVSHEDPEVKFNWYVDGVEVHNAKTKPREEQYNSTYRVVSVLTVLHQDWLNGKEYKCKVSNKALPAPIEKTISKAKGQPREPQVYTLPPCREEMTKNQVSLWCLVKGFYPSDIAVEWESNGQPENNYKTTPPVLDSDGSFFLYSKLTVDKSRWQQGNVFSCSVMHEALHNHYTQKSLSLSPGK

SEQ ID NO: 7 - protein, 450 aa, Artificial Sequence
  >SEQID7
EVQLVESGGGLVQPGGSLRLSCAASGFNIKDTYIHWVRQAPGKGLEWVGWINTYTGEPTYAADFKRRFTFSLDTSKSTAYLQMNSLRAEDTAVYYCSRWGGDGFYAMDYWGQGTLVTVSSASTKGPSVFPLAPSSKSTSGGTAALGCLVKDYFPEPVTVSWNSGALTSGVHTFPAVLQSSGLYSLSSVVTVPSSSLGTQTYICNVNHKPSNTKVDKKVEPKSCDKTHTCPPCPAPELLGGPSVFLFPPKPKDTLMISRTPEVTCVVVDVSHEDPEVKFNWYVDGVEVHNAKTKPREEQYNSTYRVVSVLTVLHQDWLNGKEYKCKVSNKALPAPIEKTISKAKGQPREPQVCTLPPSREEMTKNQVSLSCAVKGFYPSDIAVEWESNGQPENNYKTTPPVLDSDGSFFLVSKLTVDKSRWQQGNVFSCSVMHEALHNHYTQKSLSLSPGK

SEQ ID NO: 8 - protein, 450 aa, Artificial Sequence
  >SEQID8
QVQLVESGGGLVQPGGSLRLSCAASGFNIKDTYIHWVRQAPGKGLEWVARVIWYDGSKRYYADSVKGRFTISRDNSKNTLFLQMNSLRAEDTAVYYCSRWGGDGFYAMDYWGQGTLVTVSSASTKGPSVFPLAPSSKSTSGGTAALGCLVKDYFPEPVTVSWNSGALTSGVHTFPAVLQSSGLYSLSSVVTVPSSSLGTQTYICNVNHKPSNTKVDKKVEPKSCDKTHTCPPCPAPELLGGPSVFLFPPKPKDTLMISRTPEVTCVVVDVSHEDPEVKFNWYVDGVEVHNAKTKPREEQYNSTYRVVSVLTVLHQDWLNGKEYKCKVSNKALPAPIEKTISKAKGQPREPQVYTLPPSREEMTKNQVSLTCLVKGFYPSDIAVEWESNGQPENNYKTTPPVLDSDGSFFLYSKLTVDKSRWQQGNVFSCSVMHEALHNHYTQKSLSLSPG

SEQ ID NO: 9 - protein, 214 aa, Artificial Sequence
  >SEQID9
DIQMTQSPSSLSASVGDRVTITCRASQDVNTAVAWYQQKPGKAPKLLIYDASNRATGIPARFSGSGSGTDFTLTISSLQPEDFATYYCQQHYTTPPTFGQGTKVEIKRTVAAPSVFIFPPSDEQLKSGTASVVCLLNNFYPREAKVQWKVDNALQSGNSQESVTEQDSKDSTYSLSSTLTLSKADYEKHKVYACEVTHQGLSSPVTKSFNRGEC

SEQ ID NO: 10 - protein, 450 aa, Artificial Sequence
  >SEQID10
QVQLKQSGPGLVQPSQSLSITCTVSGFSLTNYGVHWVRQAPGKGLEWVGWINTYTGEPTYAADFKRRFTFSLDTSKSTAYLKMNSLQSNDTAIYYCARALTYYDYEFAYWGQGTLVTVSAASTKGPSVFPLAPSSKSTSGGTAALGCLVKDYFPEPVTVSWNSGALTSGVHTFPAVLQSSGLYSLSSVVTVPSSSLGTQTYICNVNHKPSNTKVDKKVEPKSCDKTHTCPPCPAPELLGGPSVFLFPPKPKDTLMISRTPEVTCVVVDVSHEDPEVKFNWYVDGVEVHNAKTKPREEQYNSTYRVVSVLTVLHQDWLNGKEYKCKVSNKALPAPIEKTISKAKGQPREPQVYTLPPSRDELTKNQVSLTCLVKGFYPSDIAVEWESNGQPENNYKTTPPVLDSDGSFFLYSKLTVDKSRWQQGNVFSCSVMHEALHNHYTQKSLSLSPGK

SEQ ID NO: 11 - protein, 449 aa, Artificial Sequence
  >SEQID11
QVQLVESGGGLVQPGGSLRLSCAASGFNIKDTYIHWVRQAPGKGLEWVGWINTYTGEPTYAADFKRRFTFSLDTSKSTAYLQMNSLRAEDTAVYYCSRWGGDGFYAMDYWGQGTLVTVSSASTKGPSVFPLAPSSKSTSGGTAALGCLVKDYFPEPVTVSWNSGALTSGVHTFPAVLQSSGLYSLSSVVTVPSSSLGTQTYICNVNHKPSNTKVDKKVEPKSCDKTHTCPPCPAPELLGGPSVFLFPPKPKDTLMISRTPEVTCVVVDVSHEDPEVKFNWYVDGVEVHNAKTKPREEQYNSTYRVVSVLTVLHQDWLNGKEYKCKVSNKALPAPIEKTISKAKGQPREPQVYTLPPSREEMTKNQVSLTCLVKGFYPSDIAVEWESNGQPENNYKTTPPVLDSDGSFFLYSKLTVDKSRWQQGNVFSCSVMHEALHNHYTQKSLSLSPG

SEQ ID NO: 12 - protein, 214 aa, Artificial Sequence; identical to SEQ ID NO: 9
  >SEQID12

SEQ ID NO: 13 - protein, 449 aa, Artificial Sequence
  >SEQID13
QVQLKQSGPGLVQPSQSLSITCTVSGFSLTNYGVHWVRQSPGKGLEWLGVIWSGGNTDYNTPFTSRLSINKDNSKSQVFFKMNSLQSNDTAIYYCARALTYYDYEFAYWGQGTLVTVSAASTKGPSVFPLAPSSKSTSGGTAALGCLVKDYFPEPVTVSWNSGALTSGVHTFPAVLQSSGLYSLSSVVTVPSSSLGTQTYICNVNHKPSNTKVDKRVEPKSCDKTHTCPPCPAPELLGGPSVFLFPPKPKDTLMISRTPEVTCVVVDVSHEDPEVKFNWYVDGVEVHNAKTKPREEQYNSTYRVVSVLTVLHQDWLNGKEYKCKVSNKALPAPIEKTISKAKGQPREPQVYTLPPSREEMTKNQVSLTCLVKGFYPSDIAVEWESNGQPENNYKTTPPVLDSDGSFFLYSKLTVDKSRWQQGNVFSCSVMHEALHNHYTQKSLSLSPGK

SEQ ID NO: 14 - protein, 214 aa, Artificial Sequence
  >SEQID14
DILLTQSPVILSVSPGERVSFSCRASQSIGTNIHWYQQRTNGSPRLLIKYASESISGIPSRFSGSGSGTDFTLSINSVESEDIADYYCQQNNNWPTTFGAGTKLELKRTVAAPSVFIFPPSDEQLKSGTASVVCLLNNFYPREAKVQWKVDNALQSGNSQESVTEQDSKDSTYSLSSTLTLSKADYEKHKVYACEVTHQGLSSPVTKSFNRGEC

SEQ ID NO: 15 - protein, 453 aa, Artificial Sequence
  >SEQID15
EVQLVESGGGLVQPGGSLRLSCAASGYTFTNYGMNWVRQAPGKGLEWVGWINTYTGEPTYAADFKRRFTFSLDTSKSTAYLQMNSLRAEDTAVYYCAKYPHYYGSSHWYFDVWGQGTLVTVSSASTKGPSVFPLAPSSKSTSGGTAALGCLVKDYFPEPVTVSWNSGALTSGVHTFPAVLQSSGLYSLSSVVTVPSSSLGTQTYICNVNHKPSNTKVDKKVEPKSCDKTHTCPPCPAPELLGGPSVFLFPPKPKDTLMISRTPEVTCVVVDVSHEDPEVKFNWYVDGVEVHNAKTKPREEQYNSTYRVVSVLTVLHQDWLNGKEYKCKVSNKALPAPIEKTISKAKGQPREPQVYTLPPSREEMTKNQVSLTCLVKGFYPSDIAVEWESNGQPENNYKTTPPVLDSDGSFFLYSKLTVDKSRWQQGNVFSCSVMHEALHNHYTQKSLSLSPGK

SEQ ID NO: 16 - protein, 214 aa, Artificial Sequence
  >SEQID16
DIQMTQSPSSLSASVGDRVTITCSASQDISNYLNWYQQKPGKAPKVLIYFTSSLHSGVPSRFSGSGSGTDFTLTISSLQPEDFATYYCQQYSTVPWTFGQGTKVEIKRTVAAPSVFIFPPSDEQLKSGTASVVCLLNNFYPREAKVQWKVDNALQSGNSQESVTEQDSKDSTYSLSSTLTLSKADYEKHKVYACEVTHQGLSSPVTKSFNRGEC

SEQ ID NO: 17 - protein, 449 aa, Artificial Sequence
  >SEQID17
EVQLVESGGGLVQPGGSLRLSCAASGFNIKDTYIHWVRQAPGKGLEWVARIYPTNGYTRYADSVKGRFTISADTSKNTAYLQMNSLRAEDTAVYYCSRWGGDGFYAMDYWGQGTLVTVSSASTKGPSVFPLAPSSKSTSGGTAALGCLVKDYFPEPVTVSWNSGALTSGVHTFPAVLQSSGLYSLSSVVTVPSSSLGTQTYICNVNHKPSNTKVDKKVEPKSCDKTHTCPPCPAPELLGGPSVFLFPPKPKDTLMISRTPEVTCVVVDVSHEDPEVKFNWYVDGVEVHNAKTKPREEQYNSTYRVVSVLTVLHQDWLNGKEYKCKVSNKALPAPIEKTISKAKGQPREPQVYTLPPSREEMTKNQVSLTCLVKGFYPSDIAVEWESNGQPENNYKTTPPVLDSDGSFFLYSKLTVDKSRWQQGNVFSCSVMHEALHNHYTQKSLSLSPG

SEQ ID NO: 18 - protein, 214 aa, Artificial Sequence; identical to SEQ ID NO: 5
  >SEQID18

SEQ ID NO: 19 - protein, 440 aa, Artificial Sequence
  >SEQID19
QVQLVESGGGVVQPGRSLRLDCKASGITFSNSGMHWVRQAPGKGLEWVAVIWYDGSKRYYADSVKGRFTISRDNSKNTLFLQMNSLRAEDTAVYYCATNDDYWGQGTLVTVSSASTKGPSVFPLAPCSRSTSESTAALGCLVKDYFPEPVTVSWNSGALTSGVHTFPAVLQSSGLYSLSSVVTVPSSSLGTKTYTCNVDHKPSNTKVDKRVESKYGPPCPPCPAPEFLGGPSVFLFPPKPKDTLMISRTPEVTCVVVDVSQEDPEVQFNWYVDGVEVHNAKTKPREEQFNSTYRVVSVLTVLHQDWLNGKEYKCKVSNKGLPSSIEKTISKAKGQPREPQVYTLPPSQEEMTKNQVSLTCLVKGFYPSDIAVEWESNGQPENNYKTTPPVLDSDGSFFLYSRLTVDKSRWQEGNVFSCSVMHEALHNHYTQKSLSLSLGK

SEQ ID NO: 20 - protein, 214 aa, Artificial Sequence
  >SEQID20
EIVLTQSPATLSLSPGERATLSCRASQSVSSYLAWYQQKPGQAPRLLIYDASNRATGIPARFSGSGSGTDFTLTISSLEPEDFAVYYCQQSSNWPRTFGQGTKVEIKRTVAAPSVFIFPPSDEQLKSGTASVVCLLNNFYPREAKVQWKVDNALQSGNSQESVTEQDSKDSTYSLSSTLTLSKADYEKHKVYACEVTHQGLSSPVTKSFNRGEC

SEQ ID NO: 21 - protein, 450 aa, Artificial Sequence
  >SEQID21
EVKLEESGGGLVQPGGSMKLSCVASGFIFSNHWMNWVRQSPEKGLEWVAEIRSKSINSATHYAESVKGRFTISRDDSKSAVYLQMTDLRTEDTGVYYCSRNYYGSTYDYWGQGTTLTVSSASTKGPSVFPLAPSSKSTSGGTAALGCLVKDYFPEPVTVSWNSGALTSGVHTFPAVLQSSGLYSLSSVVTVPSSSLGTQTYICNVNHKPSNTKVDKKVEPKSCDKTHTCPPCPAPELLGGPSVFLFPPKPKDTLMISRTPEVTCVVVDVSHEDPEVKFNWYVDGVEVHNAKTKPREEQYNSTYRVVSVLTVLHQDWLNGKEYKCKVSNKALPAPIEKTISKAKGQPREPQVYTLPPSRDELTKNQVSLTCLVKGFYPSDIAVEWESNGQPENNYKTTPPVLDSDGSFFLYSKLTVDKSRWQQGNVFSCSVMHEALHNHYTQKSLSLSPGK

SEQ ID NO: 22 - protein, 214 aa, Artificial Sequence
  >SEQID22
DILLTQSPAILSVSPGERVSFSCRASQFVGSSIHWYQQRTNGSPRLLIKYASESMSGIPSRFSGSGSGTDFTLSINTVESEDIADYYCQQSHSWPFTFGSGTNLEVKRTVAAPSVFIFPPSDEQLKSGTASVVCLLNNFYPREAKVQWKVDNALQSGNSQESVTEQDSKDSTYSLSSTLTLSKADYEKHKVYACEVTHQGLSSPVTKSFNRGEC

SEQ ID NO: 23 - protein, 451 aa, Artificial Sequence
  >SEQID23
EVQLVESGGGLVQPGRSLRLSCAASGFTFDDYAMHWVRQAPGKGLEWVSAITWNSGHIDYADSVEGRFTISRDNAKNSLYLQMNSLRAEDTAVYYCAKVSYLSTASSLDYWGQGTLVTVSSASTKGPSVFPLAPSSKSTSGGTAALGCLVKDYFPEPVTVSWNSGALTSGVHTFPAVLQSSGLYSLSSVVTVPSSSLGTQTYICNVNHKPSNTKVDKKVEPKSCDKTHTCPPCPAPELLGGPSVFLFPPKPKDTLMISRTPEVTCVVVDVSHEDPEVKFNWYVDGVEVHNAKTKPREEQYNSTYRVVSVLTVLHQDWLNGKEYKCKVSNKALPAPIEKTISKAKGQPREPQVYTLPPSRDELTKNQVSLTCLVKGFYPSDIAVEWESNGQPENNYKTTPPVLDSDGSFFLYSKLTVDKSRWQQGNVFSCSVMHEALHNHYTQKSLSLSPGK

SEQ ID NO: 24 - protein, 214 aa, Artificial Sequence
  >SEQID24
DIQMTQSPSSLSASVGDRVTITCRASQGIRNYLAWYQQKPGKAPKLLIYAASTLQSGVPSRFSGSGSGTDFTLTISSLQPEDVATYYCQRYNRAPYTFGQGTKVEIKRTVAAPSVFIFPPSDEQLKSGTASVVCLLNNFYPREAKVQWKVDNALQSGNSQESVTEQDSKDSTYSLSSTLTLSKADYEKHKVYACEVTHQGLSSPVTKSFNRGEC

SEQ ID NO: 25 - protein, 229 aa, Artificial Sequence
  >SEQID25
EVQLVESGGGLVQPGGSLRLSCAASGYVFTDYGMNWVRQAPGKGLEWMGWINTYIGEPIYADSVKGRFTFSLDTSKSTAYLQMNSLRAEDTAVYYCARGYRSYAMDYWGQGTLVTVSSASTKGPSVFPLAPSSKSTSGGTAALGCLVKDYFPEPVTVSWNSGALTSGVHTFPAVLQSSGLYSLSSVVTVPSSSLGTQTYICNVNHKPSNTKVDKKVEPKSCDKTHTCAA

SEQ ID NO: 26 - protein, 214 aa, Artificial Sequence
  >SEQID26
DIQMTQSPSSLSASVGDRVTITCKASQNVGTNVAWYQQKPGKAPKALIYSASFLYSGVPYRFSGSGSGTDFTLTISSLQPEDFATYYCQQYNIYPLTFGQGTKVEIKRTVAAPSVFIFPPSDEQLKSGTASVVCLLNNFYPREAKVQWKVDNALQSGNSQESVTEQDSKDSTYSLSSTLTLSKADYEKHKVYACEVTHQGLSSPVTKSFNRGEC

SEQ ID NO: 27 - protein, 457 aa, Artificial Sequence
  >SEQID27
QVQLVESGGGVVQPGRSLRLSCAASGFIFSSYAMHWVRQAPGNGLEWVAFMSYDGSNKKYADSVKGRFTISRDNSKNTLYLQMNSLRAEDTAVYYCARDRGIAAGGNYYYYGMDVISSQGTTVTVSSASTKGPSVFPLAPSSKSTSGGTAALGCLVKDYFPEPVTVSWNSGALTSGVHTFPAVLQSSGLYSLSSVVTVPSSSLGTQTYICNVNHKPSNTKVDKKVEPKSCDKTHTCPPCPAPELLGGPSVFLFPPKPKDTLMISRTPEVTCVVVDVSHEDPEVKFNWYVDGVEVHNAKTKPREEQYNSTYRVVSVLTVLHQDWLNGKEYKCKVSNKALPAPIEKTISKAKGQPREPQVYTLPPSRDELTKNQVSLTCLVKGFYPSDIAVEWESNGQPENNYKTTPPVLDSDGSFFLYSKLTVDKSRWQQGNVFSCSVMHEALHNHYTQKSLSLSPGK

SEQ ID NO: 28 - protein, 215 aa, Artificial Sequence
  >SEQID28
EIVLTQSPATLSLSPGERATLSCRASQSVYSYLAWYQQKPGQAPRLLIYDASNRATGIPARFSGSGSGTDFTLTISSLEPEDFAVYYCQQRSNWPPFTFGPGTKVDIKRTVAAPSVFIFPPSDEQLKSGTASVVCLLNNFYPREAKVQWKVDNALQSGNSQESVTEQDSKDSTYSLSSTLTLSKADYEKHKVYACEVTHQGLSSPVTKSFNRGEC

SEQ ID NO: 29 - protein, 451 aa, Artificial Sequence
  >SEQID29
QVQLQQPGAELVKPGASVKMSCKASGYTFTSYNMHWVKQTPGRGLEWIGAIYPGNGDTSYNQKFKGKATLTADKSSSTAYMQLSSLTSEDSAVYYCARSTYYGGDWYFNVWGAGTTVTVSAASTKGPSVFPLAPSSKSTSGGTAALGCLVKDYFPEPVTVSWNSGALTSGVHTFPAVLQSSGLYSLSSVVTVPSSSLGTQTYICNVNHKPSNTKVDKKVEPKSCDKTHTCPPCPAPELLGGPSVFLFPPKPKDTLMISRTPEVTCVVVDVSHEDPEVKFNWYVDGVEVHNAKTKPREEQYNSTYRVVSVLTVLHQDWLNGKEYKCKVSNKALPAPIEKTISKAKGQPREPQVYTLPPSRDELTKNQVSLTCLVKGFYPSDIAVEWESNGQPENNYKTTPPVLDSDGSFFLYSKLTVDKSRWQQGNVFSCSVMHEALHNHYTQKSLSLSPGK

SEQ ID NO: 30 - protein, 213 aa, Artificial Sequence
  >SEQID30
QIVLSQSPAILSASPGEKVTMTCRASSSVSYIHWFQQKPGSSPKPWIYATSNLASGVPVRFSGSGSGTSYSLTISRVEAEDAATYYCQQWTSNPPTFGGGTKLEIKRTVAAPSVFIFPPSDEQLKSGTASVVCLLNNFYPREAKVQWKVDNALQSGNSQESVTEQDSKDSTYSLSSTLTLSKADYEKHKVYACEVTHQGLSSPVTKSFNRGEC

SEQ ID NO: 31 - protein, 457 aa, Artificial Sequence
  >SEQID31
EVQLVESGGGLVQPGGSLRLSCAASGFTFSNYWMNWVRQAPGKGLEWVAAINQDGSEKYYVGSVKGRFTISRDNAKNSLYLQMNSLRVEDTAVYYCVRDYYDILTDYYIHYWYFDLWGRGTLVTVSSASTKGPSVFPLAPSSKSTSGGTAALGCLVKDYFPEPVTVSWNSGALTSGVHTFPAVLQSSGLYSLSSVVTVPSSSLGTQTYICNVNHKPSNTKVDKRVEPKSCDKTHTCPPCPAPELLGGPSVFLFPPKPKDTLMISRTPEVTCVVVDVSHEDPEVKFNWYVDGVEVHNAKTKPREEQYNSTYRVVSVLTVLHQDWLNGKEYKCKVSNKALPAPIEKTISKAKGQPREPQVYTLPPSREEMTKNQVSLTCLVKGFYPSDIAVEWESNGQPENNYKTTPPVLDSDGSFFLYSKLTVDKSRWQQGNVFSCSVMHEALHNHYTQKSLSLSPGK

SEQ ID NO: 32 - protein, 215 aa, Artificial Sequence
  >SEQID32
EIVLTQSPGTLSLSPGERATLSCRASQSVSSSYLAWYQQKPGQAPRLLIYGASSRATGIPDRFSGSGSGTDFTLTISRLEPEDFAVYYCQQYGSSPCTFGQGTRLEIKRTVAAPSVFIFPPSDEQLKSGTASVVCLLNNFYPREAKVQWKVDNALQSGNSQESVTEQDSKDSTYSLSSTLTLSKADYEKHKVYACEVTHQGLSSPVTKSFNRGEC

SEQ ID NO: 33 - protein, 448 aa, Artificial Sequence
  >SEQID33
QVQLVESGGGVVQPGRSLRLSCAASGFTFSSYTMHWVRQAPGKGLEWVTFISYDGNNKYYADSVKGRFTISRDNSKNTLYLQMNSLRAEDTAIYYCARTGWLGPFDYWGQGTLVTVSSASTKGPSVFPLAPSSKSTSGGTAALGCLVKDYFPEPVTVSWNSGALTSGVHTFPAVLQSSGLYSLSSVVTVPSSSLGTQTYICNVNHKPSNTKVDKRVEPKSCDKTHTCPPCPAPELLGGPSVFLFPPKPKDTLMISRTPEVTCVVVDVSHEDPEVKFNWYVDGVEVHNAKTKPREEQYNSTYRVVSVLTVLHQDWLNGKEYKCKVSNKALPAPIEKTISKAKGQPREPQVYTLPPSRDELTKNQVSLTCLVKGFYPSDIAVEWESNGQPENNYKTTPPVLDSDGSFFLYSKLTVDKSRWQQGNVFSCSVMHEALHNHYTQKSLSLSPGK

SEQ ID NO: 34 - protein, 215 aa, Artificial Sequence
  >SEQID34
EIVLTQSPGTLSLSPGERATLSCRASQSVGSSYLAWYQQKPGQAPRLLIYGAFSRATGIPDRFSGSGSGTDFTLTISRLEPEDFAVYYCQQYGSSPWTFGQGTKVEIKRTVAAPSVFIFPPSDEQLKSGTASVVCLLNNFYPREAKVQWKVDNALQSGNSQESVTEQDSKDSTYSLSSTLTLSKADYEKHKVYACEVTHQGLSSPVTKSFNRGEC

SEQ ID NO: 35 - protein, 33 aa, Artificial Sequence
  >SEQID35
QSGPGLVQPSQSLSITCTVSGFSLTNYGVHWVR

SEQ ID NO: 36 - protein, 23 aa, Artificial Sequence
  >SEQID36
GLEWLGVIWSGGNTDYNTPFTSR

SEQ ID NO: 37 - protein, 28 aa, Artificial Sequence
  >SEQID37
ARALTYYDYEFAYWGQGTLVTVSAASTK

SEQ ID NO: 38 - protein, 15 aa, Artificial Sequence
  >SEQID38
ASQSIGTNIHWYQQR

SEQ ID NO: 39 - protein, 12 aa, Artificial Sequence
  >SEQID39
YASESISGIPSR

SEQ ID NO: 40 - protein, 42 aa, Artificial Sequence
  >SEQID40
FSGSGSGTDFTLSINSVESEDIADYYCQQNNNWPTTFGAGTK

SEQ ID NO: 41 - protein, 19 aa, Artificial Sequence
  >SEQID41
LSCAASGYTFTNYGMNWVR

SEQ ID NO: 42 - protein, 22 aa, Artificial Sequence
  >SEQID42
GLEWVGWINTYTGEPTYAADFK

SEQ ID NO: 43 - protein, 9 aa, Artificial Sequence
  >SEQID43
FTFSLDTSK

SEQ ID NO: 44 - protein, 11 aa, Artificial Sequence
  >SEQID44
AEDTAVYYCAK

SEQ ID NO: 45 - protein, 31 aa, Artificial Sequence
  >SEQID45
AKYPHYYGSSHWYFDVWGQGTLVTVSSASTK

SEQ ID NO: 46 - protein, 21 aa, Artificial Sequence
  >SEQID46
VTITCSASQDISNYLNWYQQK

SEQ ID NO: 47 - protein, 16 aa, Artificial Sequence
  >SEQID47
VLIYFTSSLHSGVPSR

SEQ ID NO: 48 - protein, 42 aa, Artificial Sequence
  >SEQID48
FSGSGSGTDFTLTISSLQPEDFATYYCQQYSTVPWTFGQGTK

SEQ ID NO: 49 - protein, 15 aa, Artificial Sequence
  >SEQID49
ASGITFSNSGMHWVR

SEQ ID NO: 50 - protein, 14 aa, Artificial Sequence
  >SEQID50
GLEWVAVIWYDGSK

SEQ ID NO: 51 - protein, 30 aa, Artificial Sequence
  >SEQID51
AEDTAVYYCATNDDYWGQGTLVTVSSASTK

SEQ ID NO: 52 - protein, 15 aa, Artificial Sequence
  >SEQID52
ASQSVSSYLAWYQQK

SEQ ID NO: 53 - protein, 9 aa, Artificial Sequence
  >SEQID53
LLIYDASNR

SEQ ID NO: 54 - protein, 36 aa, Artificial Sequence
  >SEQID54
FSGSGSGTDFTLTISSLEPEDFAVYYCQQSSNWPRT

SEQ ID NO: 55 - protein, 15 aa, Artificial Sequence
  >SEQID55
ASGYTFTSYNMHWVK

SEQ ID NO: 56 - protein, 20 aa, Artificial Sequence
  >SEQID56
GLEWIGAIYPGNGDTSYNQK

SEQ ID NO: 57 - protein, 7 aa, Artificial Sequence
  >SEQID57
ATLTADK

SEQ ID NO: 58 - protein, 24 aa, Artificial Sequence
  >SEQID58
SSSTAYMQLSSLTSEDSAVYYCAR

SEQ ID NO: 59 - protein, 29 aa, Artificial Sequence
  >SEQID59
ARSTYYGGDWYFNVWGAGTTVTVSAASTK

SEQ ID NO: 60 - protein, 14 aa, Artificial Sequence
  >SEQID60
ASSSVSYIHWFQQK

SEQ ID NO: 61 - protein, 16 aa, Artificial Sequence
  >SEQID61
PWIYATSNLASGVPVR

SEQ ID NO: 62 - protein, 26 aa, Artificial Sequence
  >SEQID62
VEAEDAATYYCQQWTSNPPTFGGGTK

SEQ ID NO: 63 - protein, 19 aa, Artificial Sequence
  >SEQID63
LSCAASGFTFSNYWMNWVR

SEQ ID NO: 64 - protein, 15 aa, Artificial Sequence
  >SEQID64
GLEWVAAINQDGSEK

SEQ ID NO: 65 - protein, 11 aa, Artificial Sequence
  >SEQID65
VEDTAVYYCVR

SEQ ID NO: 66 - protein, 22 aa, Artificial Sequence
  >SEQID66
RDYYDILTDYYIHYWYFDLWGR

SEQ ID NO: 67 - protein, 16 aa, Artificial Sequence
  >SEQID67
ASQSVSSSYLAWYQQK

SEQ ID NO: 68 - protein, 9 aa, Artificial Sequence
  >SEQID68
LLIYGASSR

SEQ ID NO: 69 - protein, 26 aa, Artificial Sequence
  >SEQID69
LEPEDFAVYYCQQYGSSPCTFGQGTR

SEQ ID NO: 70 - protein, 19 aa, Artificial Sequence
  >SEQID70
LSCAASGFTFSSYTMHWVR

SEQ ID NO: 71 - protein, 15 aa, Artificial Sequence
  >SEQID71
GLEWVTFISYDGNNK

SEQ ID NO: 72 - protein, 11 aa, Artificial Sequence
  >SEQID72
AEDTAIYYCAR

SEQ ID NO: 73 - protein, 26 aa, Artificial Sequence
  >SEQID73
ARTGWLGPFDYWGQGTLVTVSSASTK

SEQ ID NO: 74 - protein, 16 aa, Artificial Sequence
  >SEQID74
ASQSVGSSYLAWYQQK

SEQ ID NO: 75 - protein, 9 aa, Artificial Sequence
  >SEQID75
LLIYGAFSR

SEQ ID NO: 76 - protein, 26 aa, Artificial Sequence
  >SEQID76
LEPEDFAVYYCQQYGSSPWTFGQGTK

SEQ ID NO: 77 - protein, 8 aa, Artificial Sequence
  >SEQID77
GITFSNSG

SEQ ID NO: 78 - protein, 17 aa, Artificial Sequence
  >SEQID78
VIWYDGSKRYYADSVKG

SEQ ID NO: 79 - protein, 6 aa, Artificial Sequence
  >SEQID79
ATNDDY

SEQ ID NO: 80 - protein, 6 aa, Artificial Sequence
  >SEQID80
QSVSSY

SEQ ID NO: 81 - skipped

SEQ ID NO: 82 - protein, 9 aa, Artificial Sequence
  >SEQID82
QQSSNWPRT

SEQ ID NO: 83 - protein, 8 aa, Artificial Sequence
  >SEQID83
GFSLTNYG

SEQ ID NO: 84 - protein, 7 aa, Artificial Sequence
  >SEQID84
IWSGGNT

SEQ ID NO: 85 - protein, 13 aa, Artificial Sequence
  >SEQID85
ARALTYYDYEFAY

SEQ ID NO: 86 - protein, 6 aa, Artificial Sequence
  >SEQID86
QSIGTN

SEQ ID NO: 87 - skipped

SEQ ID NO: 88 - protein, 9 aa, Artificial Sequence
  >SEQID88
QQNNNWPTT

SEQ ID NO: 89 - protein, 8 aa, Artificial Sequence
  >SEQID89
GYTFTNYG

SEQ ID NO: 90 - protein, 11 aa, Artificial Sequence
  >SEQID90
GWINTYTGEPT

SEQ ID NO: 91 - protein, 17 aa, Artificial Sequence
  >SEQID91
AKYPHYYGSSHWYFDVW

SEQ ID NO: 92 - protein, 6 aa, Artificial Sequence
  >SEQID92
QDISNY

SEQ ID NO: 93 - skipped

SEQ ID NO: 94 - protein, 8 aa, Artificial Sequence
  >SEQID94
QQYSTVPW

SEQ ID NO: 95 - protein, 8 aa, Artificial Sequence
  >SEQID95
GYTFTSYN

SEQ ID NO: 96 - protein, 9 aa, Artificial Sequence
  >SEQID96
IYPGNGDTS

SEQ ID NO: 97 - protein, 14 aa, Artificial Sequence
  >SEQID97
ARSTYYGGDWYFNV

SEQ ID NO: 98 - protein, 5 aa, Artificial Sequence
  >SEQID98
SSVSY

SEQ ID NO: 99 - skipped

SEQ ID NO: 100 - protein, 9 aa, Artificial Sequence
  >SEQID100
QQWTSNPPT

SEQ ID NO: 101 - protein, 8 aa, Artificial Sequence
  >SEQID101
GFTFSNYW

SEQ ID NO: 102 - protein, 9 aa, Artificial Sequence
  >SEQID102
AINQDGSEK

SEQ ID NO: 103 - protein, 19 aa, Artificial Sequence
  >SEQID103
RDYYDILTDYYIHYWYFDL

SEQ ID NO: 104 - protein, 7 aa, Artificial Sequence
  >SEQID104
QSVSSSY

SEQ ID NO: 105 - skipped

SEQ ID NO: 106 - protein, 8 aa, Artificial Sequence
  >SEQID106
QQYGSSPC

SEQ ID NO: 107 - protein, 8 aa, Artificial Sequence
  >SEQID107
GFTFSSYT

SEQ ID NO: 108 - protein, 10 aa, Artificial Sequence
  >SEQID108
TFISYDGNNK

SEQ ID NO: 109 - protein, 11 aa, Artificial Sequence
  >SEQID109
ARTGWLGPFDY

SEQ ID NO: 110 - protein, 7 aa, Artificial Sequence
  >SEQID110
QSVGSSY

SEQ ID NO: 111 - skipped

SEQ ID NO: 112 - protein, 9 aa, Artificial Sequence
  >SEQID112
QQYGSSPWT

SEQ ID NO: 113 - protein, 448 aa, Artificial Sequence
  >SEQID113
EVQLVESGGGLVQPGGSLRLSCKASGITFSNSGMHWVRQAPGKGLEWLGVIWSGGNTDYNTPFTSRFTISADTSKNTAYLQMNSLRAEDTAVYYCSRWGGDGFYAMDYWGQGTLVTVSSASTKGPSVFPLAPSSKSTSGGTAALGCLVKDYFPEPVTVSWNSGALTSGVHTFPAVLQSSGLYSLSSVVTVPSSSLGTQTYICNVNHKPSNTKVDKKVEPKSCDKTHTCPPCPAPELLGGPSVFLFPPKPKDTLMISRTPEVTCVVVDVSHEDPEVKFNWYVDGVEVHNAKTKPREEQYNSTYRVVSVLTVLHQDWLNGKEYKCKVSNKALPAPIEKTISKAKGQPREPQVYTLPPSREEMTKNQVSLTCLVKGFYPSDIAVEWESNGQPENNYKTTPPVLDSDGSFFLYSKLTVDKSRWQQGNVFSCSVMHEALHNHYTQKSLSLSPG

SEQ ID NO: 114 - protein, 214 aa, Artificial Sequence
  >SEQID114
DIQMTQSPSSLSASVGDRVTITCRASQSVSSYLAWYQQKPGKAPKLLIKYASESISGIPSRFSGSRSGTDFTLTISSLQPEDFATYYCQQHYTTPPTFGQGTKVEIKRTVAAPSVFIFPPSDEQLKSGTASVVCLLNNFYPREAKVQWKVDNALQSGNSQESVTEQDSKDSTYSLSSTLTLSKADYEKHKVYACEVTHQGLSSPVTKSFNRGEC

SEQ ID NO: 115 - protein, 450 aa, Artificial Sequence
  >SEQID115
EVQLVESGGGLVQPGGSLRLSCAASGFNIKDTYIHWVRQAPGKGLEWVAVIWYDGSKRYYADSVKGRFTISADTSKNTAYLQMNSLRAEDTAVYYCSRWGGDGFYAMDYWGQGTLVTVSSASTKGPSVFPLAPSSKSTSGGTAALGCLVKDYFPEPVTVSWNSGALTSGVHTFPAVLQSSGLYSLSSVVTVPSSSLGTQTYICNVNHKPSNTKVDKKVEPKSCDKTHTCPPCPAPELLGGPSVFLFPPKPKDTLMISRTPEVTCVVVDVSHEDPEVKFNWYVDGVEVHNAKTKPREEQYNSTYRVVSVLTVLHQDWLNGKEYKCKVSNKALPAPIEKTISKAKGQPREPQVYTLPPSREEMTKNQVSLTCLVKGFYPSDIAVEWESNGQPENNYKTTPPVLDSDGSFFLYSKLTVDKSRWQQGNVFSCSVMHEALHNHYTQKSLSLSPGK

SEQ ID NO: 116 - protein, 451 aa, Artificial Sequence
  >SEQID116
EVQLVESGGGLVQPGGSLRLSCAASGFNIKDTYIHWVRQAPGKPGKGLEWLGVIWSGGNTDYNTPFTSRLSINKDNSKNTAYLQMNSLRAEDTAVYYCSRWGGDGFYAMDYWGQGTLVTVSSASTKGPSVFPLAPSSKSTSGGTAALGCLVKDYFPEPVTVSWNSGALTSGVHTFPAVLQSSGLYSLSSVVTVPSSSLGTQTYICNVNHKPSNTKVDKKVEPKSCDKTHTCPPCPAPELLGGPSVFLFPPKPKDTLMISRTPEVTCVVVDVSHEDPEVKFNWYVDGVEVHNAKTKPREEQYNSTYRVVSVLTVLHQDWLNGKEYKCKVSNKALPAPIEKTISKAKGQPREPQVYTLPPSREEMTKNQVSLTCLVKGFYPSDIAVEWESNGQPENNYKTTPPVLDSDGSFFLYSKLTVDKSRWQQGNVFSCSVMHEALHNHYTQKSLSLSPG

SEQ ID NO: 117 - protein, 214 aa, Artificial Sequence
  >SEQID117
DIQMTQSPSSLSASVGDRVTLSCRASQSVSSYLAWYQQKPGKAPRLLIYDASNRATGVPSRFSGSRSGTDFTLTISSLQPEDFATYYCQQHYTTPPTFGQGTKVEIKRTVAAPSVFIFPPSDEQLKSGTASVVCLLNNFYPREAKVQWKVDNALQSGNSQESVTEQDSKDSTYSLSSTLTLSKADYEKHKVYACEVTHQGLSSPVTKSFNRGEC

SEQ ID NO: 118 - protein, 214 aa, Artificial Sequence
  >SEQID118
DIQMTQSPSSLSASVGDRVTITCRASQSIGTNIHWYQQRTNGSPRLLIKYASESISGIPSRFSGSRSGTDFTLTISSLQPEDFATYYCQQHYTTPPTFGQGTKVEIKRTVAAPSVFIFPPSDEQLKSGTASVVCLLNNFYPREAKVQWKVDNALQSGNSQESVTEQDSKDSTYSLSSTLTLSKADYEKHKVYACEVTHQGLSSPVTKSFNRGEC

SEQ ID NO: 119 - protein, 450 aa, Artificial Sequence
  >SEQID119
EVQLVESGGGLVQPGGSLRLSCAASGFNIKDTYIHWVRQAPGKGLEWVGWINTYTGEPTYAADFKRRFTFSLDTSKSTAYLQMNSLRAEDTAVYYCSRWGGDGFYAMDYWGQGTLVTVSSASTKGPSVFPLAPSSKSTSGGTAALGCLVKDYFPEPVTVSWNSGALTSGVHTFPAVLQSSGLYSLSSVVTVPSSSLGTQTYICNVNHKPSNTKVDKKVEPKSCDKTHTCPPCPAPELLGGPSVFLFPPKPKDTLMISRTPEVTCVVVDVSHEDPEVKFNWYVDGVEVHNAKTKPREEQYNSTYRVVSVLTVLHQDWLNGKEYKCKVSNKALPAPIEKTISKAKGQPREPQVYTLPPSREEMTKNQVSLTCLVKGFYPSDIAVEWESNGQPENNYKTTPPVLDSDGSFFLYSKLTVDKSRWQQGNVFSCSVMHEALHNHYTQKSLSLSPGK